European Patent Application EP 4 421 162 A1, published August 28, 2024. Title: Autoimmune disease therapeutic agent containing oligonucleotide selectively binding to IFN-γ and oligonucleotide thereof. Applicant: TAGCYX Biotechnologies Inc. The sequence listing filed with the application follows.

SEQUENCE LISTING (3 sequences)

SEQ ID NO: 1 - DNA, 48 bp, synthetic construct
  source 1..48: mol_type = other DNA
  misc_feature 28: note = n is synthetic base; Ds(7-(2-thienyl)imidazo[4,5-b]pyridine)
  misc_feature 39: note = n is synthetic base; Ds(7-(2-thienyl)imidazo[4,5-b]pyridine)
cccgcccgggtccgcgaagcggtaggtntgggctaggcngctggcggg

SEQ ID NO: 2 - DNA, 57 bp, synthetic construct
  source 1..57: mol_type = other DNA
  misc_feature 28: note = n is synthetic base; Ds(7-(2-thienyl)imidazo[4,5-b]pyridine)
  misc_feature 39: note = n is synthetic base; Ds(7-(2-thienyl)imidazo[4,5-b]pyridine)
cccgcccgggtccgcgaagcggtaggtntgggctaggcngctggcgggcgcgaagcg

SEQ ID NO: 3 - DNA, 57 bp, synthetic construct
  source 1..57: mol_type = other DNA
  misc_feature 28: note = n is synthetic base; Ds(7-(2-thienyl)imidazo[4,5-b]pyridine)
  misc_feature 39: note = n is synthetic base; Ds(7-(2-thienyl)imidazo[4,5-b]pyridine)
  misc_feature 53: note = n is a natural base or an artificial base
cccgcccgggtccgcgaagcggtaggtntgggctaggcngctggcgggcgcgnagcg